European Patent Application EP 4 703 378 A1, published March 4, 2026. Title: 改善眼部血管新生相关疾病的药物及其应用. Applicant: 南京贝思奥生物科技有限公司. The sequence listing filed with the application follows.

SEQUENCE LISTING (12 sequences)

SEQ ID NO: 1 - protein, 11 aa, synthetic construct
QASEIIHSWLA

SEQ ID NO: 2 - protein, 7 aa, synthetic construct
LASTLAS

SEQ ID NO: 3 - protein, 12 aa, synthetic construct
QNVYLASTNGAN

SEQ ID NO: 4 - protein, 6 aa, synthetic construct
DYYYMT

SEQ ID NO: 5 - protein, 16 aa, synthetic construct
FIDPDDDPYYATWAKG

SEQ ID NO: 6 - protein, 11 aa, synthetic construct
GDHNSGWGLDI

SEQ ID NO: 7 - protein, 110 aa, synthetic construct
EIVMTQSPSTLSASVGDRVIITCQASEIIHSWLAWYQQKPGKAPKLLIYLASTLASGVPSRFSGSGSGAEFTLTISSLQPDDFATYYCQNVYLASTNGANFGQGTKLTVL

SEQ ID NO: 8 - protein, 120 aa, synthetic construct
EVQLVESGGGLVQPGGSLRLSCTASGFSLTDYYYMTWVRQAPGKGLEWVGFIDPDDDPYYATWAKGRFTISRDNSKNTLYLQMNSLRAEDTAVYYCAGGDHNSGWGLDIWGQGTLVTVSS

SEQ ID NO: 9 - protein, 20 aa, synthetic construct
METHSQVFVYMLLCLSGVEG

SEQ ID NO: 10 - DNA, 330 bp, synthetic construct
  source 1..330: mol_type = other DNA
gagatcgtgatgacccagagccccagcaccctgagcgccagcgtgggcgacagggtgatcatcacctgccaggccagcgagatcatccacagctggctggcctggtaccagcagaagcccggcaaggcccccaagctgctgatctacctggccagcaccctggccagcggcgtgcccagcaggttcagcggcagcggcagcggcgccgagttcaccctgaccatcagcagcctgcagcccgacgacttcgccacctactactgccagaacgtgtacctggccagcaccaacggcgccaacttcggccagggcaccaagctgaccgtgctg

SEQ ID NO: 11 - DNA, 363 bp, synthetic construct
  source 1..363: mol_type = other DNA
gaggtgcagctggtggagagcggcggcggcctggtgcagcccggcggcagcctgaggctgagctgcaccgccagcggcttcagcctgaccgactactactacatgacctgggtgaggcaggcccccggcaagggcctggagtgggtgggcttcatcgaccccgacgacgacccctactacgccacctgggccaagggcaggttcaccatcagcagggacaacagcaagaacaccctgtacctgcagatgaacagcctgagggccgaggacaccgccgtgtactactgcgccggcggcgaccacaacagcggctggggcctggacatctggggccagggcaccctggtgaccgtgagcagctga

SEQ ID NO: 12 - DNA, 816 bp, synthetic construct
  source 1..816: mol_type = other DNA
atggagacacattctcaggtctttgtatacatgttgctgtgtttgtctggtgtcgagggcgagatcgtgatgacccagagccccagcaccctgagcgccagcgtgggcgacagggtgatcatcacctgccaggccagcgagatcatccacagctggctggcctggtaccagcagaagcccggcaaggcccccaagctgctgatctacctggccagcaccctggccagcggcgtgcccagcaggttcagcggcagcggcagcggcgccgagttcaccctgaccatcagcagcctgcagcccgacgacttcgccacctactactgccagaacgtgtacctggccagcaccaacggcgccaacttcggccagggcaccaagctgaccgtgctgggcggcggcggcggcagcggcggcggcggcagcggcggcggcggcagcggcggcggcggcagcgaggtgcagctggtggagagcggcggcggcctggtgcagcccggcggcagcctgaggctgagctgcaccgccagcggcttcagcctgaccgactactactacatgacctgggtgaggcaggcccccggcaagggcctggagtgggtgggcttcatcgaccccgacgacgacccctactacgccacctgggccaagggcaggttcaccatcagcagggacaacagcaagaacaccctgtacctgcagatgaacagcctgagggccgaggacaccgccgtgtactactgcgccggcggcgaccacaacagcggctggggcctggacatctggggccagggcaccctggtgaccgtgagcagctga